European Patent Application EP 4 115 904 A2, published January 11, 2023. Title: Anti-RSPO3 Antibodies. Applicant: National Health Research Institutes. The sequence listing filed with the application follows.

SEQUENCE LISTING (84 sequences)

SEQ ID NO: 1 - DNA, 345 bp, Artificial Sequence
  Synthetic polynucleotide
caggtgcaactgcaggagtctggggctgaactggcaaaacctggggcctcagtgaagatgtcctgcaaggcttctggccacactctaacttactactggatgcactgggtaaaacagaggcctggacagggtctggaatggattggatacattgatcctagcactggttatagtgaatacaatcaaagattcgagggcaaggccacattgactgcagacaagtcctccggcacagtctacatgcagctgagcagcctgacatctgaggactctgcggtctattactgtgcaagaaacgggccctttgcttactggggccaagggactctggtcactgtctctgcg

SEQ ID NO: 2 - protein, 115 aa, Artificial Sequence
  heavy chain variable region
QVQLQESGAELAKPGASVKMSCKASGHTLTYYWMHWVKQRPGQGLEWIGYIDPSTGYSEYNQRFEGKATLTADKSSGTVYMQLSSLTSEDSAVYYCARNGPFAYWGQGTLVTVSA

SEQ ID NO: 3 - DNA, 321 bp, Artificial Sequence
  Synthetic polynucleotide
gacaatgttctcacccagtctccagcaatcatgtctgcatctccaggggagaaggtcaccatgacctgcagtgccagctcaagtgtaaattacatgtactggtaccagcagaagccgggatcctcccccagactcctgatttatgacacatccaagctggcttccggagtccctgttcgcttcagtggcagtgggtctgggacctcttactctctcacaatcagccgaatggaggctgaagatgctgccacttattattgccagcagtggagtagttccccgctcacgttcggtgttggggccaagctggaaatcaaacgc

SEQ ID NO: 4 - protein, 107 aa, Artificial Sequence
  Light chain variable region
DNVLTQSPAIMSASPGEKVTMTCSASSSVNYMYWYQQKPGSSPRLLIYDTSKLASGVPVRFSGSGSGTSYSLTISRMEAEDAATYYCQQWSSSPLTFGVGAKLEIKR

SEQ ID NO: 5 - DNA, 345 bp, Artificial Sequence
  Synthetic polynucleotide
caggtccaactgcagcagtctggggcagagattgtgaggtcaggggcctcagtcaagttgtcctgcacagcttctggcttcagtattacagaatactatatacactgggtgaagcagaggcctgatcagggcctggagtggataggaatgattgatcctgagaatggtgatactgactatgccccgaagttccagggcaaggccactatgactgcagacacatcgtccaatacagtcaacctgcaactcagcagcctgacatctgaggacactgccgtctattactgtcatggaccgggcccccttgagtactggggccaaggcaccactctcacagtctcctcg

SEQ ID NO: 6 - protein, 115 aa, Artificial Sequence
  Heavy chain variable region
QVQLQQSGAEIVRSGASVKLSCTASGFSITEYYIHWVKQRPDQGLEWIGMIDPENGDTDYAPKFQGKATMTADTSSNTVNLQLSSLTSEDTAVYYCHGPGPLEYWGQGTTLTVSS

SEQ ID NO: 7 - DNA, 339 bp, Artificial Sequence
  Synthetic polynucleotide
gacattgtaatgacccaatctccactctccctgcctgtcagtcttggagatcaagcctccatctcttgtagatctagtcagagtattgtacatagtaatggaaacacttatttagaatggtacctgcagaaaccaggccagtctccaaacctcctgatctacagagtttccaaccgcttttctggggtcccagacaggttcaatggcagtggatcagggacagatttcacactcaagatcagcagagtggagcctgaggatctgggagtttattcctgctttcaagcttcacatgttccgtacacgttcggaggggggaccaagctggaaataaaacgc

SEQ ID NO: 8 - protein, 113 aa, Artificial Sequence
  Light chain variable region
DIVMTQSPLSLPVSLGDQASISCRSSQSIVHSNGNTYLEWYLQKPGQSPNLLIYRVSNRFSGVPDRFNGSGSGTDFTLKISRVEPEDLGVYSCFQASHVPYTFGGGTKLEIKR

SEQ ID NO: 9 - DNA, 351 bp, Artificial Sequence
  Synthetic polynucleotide
cagattcagcttcaggagtcaggacctggcctcgtgaaaccttctcagtctctgtctctcacctgctctgtcactggctactcaataaccagtggttattattggaattggatccggcagtttccaggaaataaactggaatggatgggctacataagttacgacggtaccaataactacaacccatctctcaaagatcgaatctccatcactcgtgacacatctatgaaccagtttttcctgaagttgaattctgtgactactgaggacacagctacatattactgttcagtcttattaatacagtacttcaatatctggggcgccggaaccacggtcaccgtctcctcg

SEQ ID NO: 10 - protein, 117 aa, Artificial Sequence
  Heavy chain variable region
QIQLQESGPGLVKPSQSLSLTCSVTGYSITSGYYWNWIRQFPGNKLEWMGYISYDGTNNYNPSLKDRISITRDTSMNQFFLKLNSVTTEDTATYYCSVLLIQYFNIWGAGTTVTVSS

SEQ ID NO: 11 - DNA, 324 bp, Artificial Sequence
  Synthetic polynuceotide
gacatccagatgacacagtctccagcctccctatctgcatctgtgggagaaaccgtcaccatcacatgtcgaacaagtgagagtgttaacaatttcttagcctggtttcaccagaaacagggaaaatctcctcaactcctggtctatcatgcaaaaaccttagcagatggtgtgtcatcaaggttcagtggcagtggatcaggaacacaatattctctcaagatcaacagcctgcagcctgaagattttgggaattattactgtcaacatttttggagtattccgtggacgttcggtggaggcaccaagctggaaatcaaacgc

SEQ ID NO: 12 - protein, 108 aa, Artificial Sequence
  Light chain variable region
DIQMTQSPASLSASVGETVTITCRTSESVNNFLAWFHQKQGKSPQLLVYHAKTLADGVSSRFSGSGSGTQYSLKINSLQPEDFGNYYCQHFWSIPWTFGGGTKLEIKR

SEQ ID NO: 13 - DNA, 351 bp, Artificial Sequence
  Synthetic polynucleotide
cagatccagctccaagagagcggccccggcctggtgaagcccagcgagagcctgagcctgacctgctcggtgaccggctacagcatcaccagcggctactactggaactggatcaggcagttccccggcaacggcctggagtggatgggctacatcagctacgacggcaccaacaactacaaccccagcctgaaggacaggatcagcatcaccagggacaccagcaagaaccagttcttcctgaagctgaacagcgtgaccgccgccgacaccgccacctactactgctcggtgctgctgatccagtacttcaacatctggggcaagggcaccaccgtgaccgtgagcagc

SEQ ID NO: 14 - protein, 117 aa, Artificial Sequence
  Heavy chain variable region
QIQLQESGPGLVKPSESLSLTCSVTGYSITSGYYWNWIRQFPGNGLEWMGYISYDGTNNYNPSLKDRISITRDTSKNQFFLKLNSVTAADTATYYCSVLLIQYFNIWGKGTTVTVSS

SEQ ID NO: 15 - DNA, 324 bp, Artificial Sequence
  Synthetic polynucleotide
gacatccagatgacccagagccccagcagcctgagcgccagcgtgggcgagagggtgaccatcacctgccgtaccagcgagagcgtgaacaacttcctggcctggttccaccagaagcccggcaagagccccaagctgctggtgtaccacgccaagaccctggccgacggcgtgagcagcaggttcagcggcagcggcagcggcacccagtacagcctgaagatcaacagcctgcaacccgaggacttcggcaactactactgccagcacttctggagcatcccctggaccttcggcggcggcaccaagctggagatcaagagg

SEQ ID NO: 16 - protein, 108 aa, Artificial Sequence
  Light chain variable region
DIQMTQSPSSLSASVGERVTITCRTSESVNNFLAWFHQKPGKSPKLLVYHAKTLADGVSSRFSGSGSGTQYSLKINSLQPEDFGNYYCQHFWSIPWTFGGGTKLEIKR

SEQ ID NO: 17 - DNA, 20 bp, Artificial Sequence
  Synthetic oligonucleotide
gacawtgttctcacccagtc

SEQ ID NO: 18 - DNA, 20 bp, Artificial Sequence
  Synthetic oligonucleotide
gacatccagatgacacagwc

SEQ ID NO: 19 - DNA, 20 bp, Artificial Sequence
  Synthetic oligonucleotide
gatrttgtgatgacccagwc

SEQ ID NO: 20 - DNA, 20 bp, Artificial Sequence
  Synthetic oligonucleotide
gacattstgmtgacccagtc

SEQ ID NO: 21 - DNA, 20 bp, Artificial Sequence
  Synthetic oligonucleotide
gatgttgtgvtgacccaaac

SEQ ID NO: 22 - DNA, 20 bp, Artificial Sequence
  Synthetic oligonucleotide
gacacaactgtgacccagtc

SEQ ID NO: 23 - DNA, 20 bp, Artificial Sequence
  Synthetic oligonucleotide
gayattktgctcactcagtc

SEQ ID NO: 24 - DNA, 20 bp, Artificial Sequence
  Synthetic oligonucleotide
gatattgtgatracccaggm

SEQ ID NO: 25 - DNA, 20 bp, Artificial Sequence
  Synthetic oligonucleotide
gacattgtaatgacccaatc

SEQ ID NO: 26 - DNA, 20 bp, Artificial Sequence
  Synthetic oligonucleotide
gacattgtgatgwcacagtc

SEQ ID NO: 27 - DNA, 20 bp, Artificial Sequence
  Synthetic oligonucleotide
gatrtccagatgamccagtc

SEQ ID NO: 28 - DNA, 20 bp, Artificial Sequence
  Synthetic oligonucleotide
gatggagaaacaacacaggc

SEQ ID NO: 29 - DNA, 20 bp, Artificial Sequence
  Synthetic oligonucleotide
gacgctgttgtgactcagga

SEQ ID NO: 30 - DNA, 20 bp, Artificial Sequence
  Synthetic oligonucleotide
gaccytgtgctcactcagtc

SEQ ID NO: 31 - DNA, 20 bp, Artificial Sequence
  Synthetic oligonucleotide
gcgtttbatttccagcttgg

SEQ ID NO: 32 - DNA, 20 bp, Artificial Sequence
  Synthetic oligonucleotide
gcgttttatttccaattttg

SEQ ID NO: 33 - DNA, 19 bp, Artificial Sequence
  Synthetic oligonucleotide
gcctaggacagtcamcytg

SEQ ID NO: 34 - DNA, 20 bp, Artificial Sequence
  Synthetic oligonucleotide
gaggttcdsctgcaacagty

SEQ ID NO: 35 - DNA, 20 bp, Artificial Sequence
  Synthetic oligonucleotide
caggtgcaamtgmagsagtc

SEQ ID NO: 36 - DNA, 20 bp, Artificial Sequence
  Synthetic oligonucleotide
gavgtgmwgctggtggagtc

SEQ ID NO: 37 - DNA, 20 bp, Artificial Sequence
  Synthetic oligonucleotide
caggttaytctgaaagagtc

SEQ ID NO: 38 - DNA, 20 bp, Artificial Sequence
  Synthetic oligonucleotide
gakgtgcagcttcagsagtc

SEQ ID NO: 39 - DNA, 20 bp, Artificial Sequence
  Synthetic oligonucleotide
cagatccagttsgygcagtc

SEQ ID NO: 40 - DNA, 20 bp, Artificial Sequence
  Synthetic oligonucleotide
cagrtccaactgcagcagyc

SEQ ID NO: 41 - DNA, 20 bp, Artificial Sequence
  Synthetic oligonucleotide
gaggtgmagctasttgagwc

SEQ ID NO: 42 - DNA, 20 bp, Artificial Sequence
  Synthetic oligonucleotide
gaagtgaagmttgaggagtc

SEQ ID NO: 43 - DNA, 20 bp, Artificial Sequence
  Synthetic oligonucleotide
gatgtgaacctggaagtgtc

SEQ ID NO: 44 - DNA, 20 bp, Artificial Sequence
  Synthetic oligonucleotide
cagatkcagcttmaggagtc

SEQ ID NO: 45 - DNA, 20 bp, Artificial Sequence
  Synthetic oligonucleotide
caggcttatctgcagcagtc

SEQ ID NO: 46 - DNA, 20 bp, Artificial Sequence
  Synthetic oligonucleotide
caggttcacctacaacagtc

SEQ ID NO: 47 - DNA, 20 bp, Artificial Sequence
  Synthetic oligonucleotide
caggtgcagcttgtagagac

SEQ ID NO: 48 - DNA, 20 bp, Artificial Sequence
  Synthetic oligonucleotide
gargtgmagctgktggagac

SEQ ID NO: 49 - DNA, 20 bp, Artificial Sequence
  Synthetic oligonucleotide
cgaggagacggtgacmgtgg

SEQ ID NO: 50 - DNA, 20 bp, Artificial Sequence
  Synthetic oligonucleotide
cgcagagacagtgaccagag

SEQ ID NO: 51 - DNA, 20 bp, Artificial Sequence
  Synthetic oligonucleotide
cgaggagactgtgagastgg

SEQ ID NO: 52 - DNA, 38 bp, Artificial Sequence
  Synthetic oligonucleotide
catgcctaggccaccatgtacaggatgcaactcctgtc

SEQ ID NO: 53 - DNA, 31 bp, Artificial Sequence
  Synthetic oligonucleotide
gggtttcatatgtcatttacccggagacagg

SEQ ID NO: 54 - DNA, 38 bp, Artificial Sequence
  Synthetic oligonucleotide
ggaagatatcccaccatgtacaggatgcaactcctgtc

SEQ ID NO: 55 - DNA, 33 bp, Artificial Sequence
  Synthetic oligonucleotide
ccttaattaactaacactctcccctgttgaagc

SEQ ID NO: 56 - DNA, 19 bp, Artificial Sequence
  Synthetic oligonucleotide
gaaggtgaaggtcggagtc

SEQ ID NO: 57 - DNA, 20 bp, Artificial Sequence
  Synthetic oligonucleotide
gaagatggtgatgggatttc

SEQ ID NO: 58 - DNA, 19 bp, Artificial Sequence
  Synthetic oligonucleotide
tgatgaccattgcctacac

SEQ ID NO: 59 - DNA, 24 bp, Artificial Sequence
  Synthetic oligonucleotide
gtaaggtttattaaagaggagaag

SEQ ID NO: 60 - DNA, 20 bp, Artificial Sequence
  Synthetic oligonucleotide
tccccaccttgaatgaagaa

SEQ ID NO: 61 - DNA, 18 bp, Artificial Sequence
  Synthetic oligonucleotide
tggtggctggtgcaaaga

SEQ ID NO: 62 - DNA, 16 bp, Artificial Sequence
  Synthetic oligonucleotide
cacccggccattgtgc

SEQ ID NO: 63 - DNA, 17 bp, Artificial Sequence
  Synthetic oligonucleotide
gcttttccctcgaccgc

SEQ ID NO: 64 - DNA, 21 bp, Artificial Sequence
  Synthetic oligonucleotide
gcattggcatcttctatggtt

SEQ ID NO: 65 - DNA, 20 bp, Artificial Sequence
  Synthetic oligonucleotide
cgccttgtccttggtagtgt

SEQ ID NO: 66 - DNA, 22 bp, Artificial Sequence
  Synthetic oligonucleotide
tccaacacctcccagtatgaca

SEQ ID NO: 67 - DNA, 22 bp, Artificial Sequence
  Synthetic oligonucleotide
tcttcaggattcgttctgtatt

SEQ ID NO: 68 - DNA, 19 bp, Artificial Sequence
  Synthetic oligonucleotide
gccaaacagtgcccagacc

SEQ ID NO: 69 - DNA, 19 bp, Artificial Sequence
  Synthetic oligonucleotide
ctctcgaccgttgtgtgcg

SEQ ID NO: 70 - DNA, 20 bp, Artificial Sequence
  Synthetic oligonucleotide
acgccagaacaacgaatacc

SEQ ID NO: 71 - DNA, 20 bp, Artificial Sequence
  Synthetic oligonucleotide
acgaccttgccatccactac

SEQ ID NO: 72 - protein, 277 aa, Artificial Sequence
  Synthetic polypeptide
  MISC_FEATURE (1)..(277): mRSPO3
MHLRLISCFFIILNFMEYIGSQNASRGRRQRRMHPNVSQGCQGGCATCSDYNGCLSCKPRLFFVLERIGMKQIGVCLSSCPSGYYGTRYPDINKCTKCKVDCDTCFNKNFCTKCKSGFYLHLGKCLDSCPEGLEANNHTMECVSIVHCEASEWSPWSPCMKKGKTCGFKRGTETRVRDILQHPSAKGNLCPPTSETRTCIVQRKKCSKGERGKKGRERKRKKLNKEERKETSSSSDSKGLESSIETPDQQENKERQQQQKRRARDKQQKSVSVSTVH

SEQ ID NO: 73 - protein, 272 aa, Artificial Sequence
  Synthetic polypeptide
  MISC_FEATURE (1)..(272): hRSPO3
MHLRLISWLFIILNFMEYIGSQNASRGRRQRRMHPNVSQGCQGGCATCSDYNGCLSCKPRLFFALERIGMKQIGVCLSSCPSGYYGTRYPDINKCTKCKADCDTCFNKNFCTKCKSGFYLHLGKCLDNCPEGLEANNHTMECVSIVHCEVSEWNPWSPCTKKGKTCGFKRGTETRVREIIQHPSAKGNLCPPTNETRKCTVQRKKCQKGERGKKGRERKRKKPNKGESKEAIPDSKSLESSKEIPEQRENKQQQKKRKVQDKQKSVSVSTVH

SEQ ID NO: 74 - protein, 10 aa, Artificial Sequence
  Synthetic polypeptide
QNASRGRRQR

SEQ ID NO: 75 - protein, 10 aa, Artificial Sequence
  Synthetic polypeptide
ASRGRRQRRM

SEQ ID NO: 76 - protein, 10 aa, Artificial Sequence
  Synthetic polypeptide
RGRRQRRMHP

SEQ ID NO: 77 - protein, 10 aa, Artificial Sequence
  Synthetic polypeptide
RRQRRMHPNV

SEQ ID NO: 78 - protein, 10 aa, Artificial Sequence
  Synthetic polypeptide
CLSCKPRLFF

SEQ ID NO: 79 - protein, 10 aa, Artificial Sequence
  Synthetic polypeptide
SCKPRLFFAL

SEQ ID NO: 80 - protein, 10 aa, Artificial Sequence
  Synthetic polypeptide
ERGKKGRERK

SEQ ID NO: 81 - protein, 10 aa, Artificial Sequence
  Synthetic polypeptide
GKKGRERKRK

SEQ ID NO: 82 - protein, 10 aa, Artificial Sequence
  Synthetic polypeptide
KGRERKRKKP

SEQ ID NO: 83 - protein, 10 aa, Artificial Sequence
  Synthetic polypeptide
RERKRKKPNK

SEQ ID NO: 84 - protein, 10 aa, Artificial Sequence
  Synthetic polypeptide
RENKQQQKKR